European Patent Specification EP 3 528 839 B1, published November 8, 2023. Title: ExPEC glycoconjugate vaccine formulations. Applicant: Janssen Vaccines & Prevention B.V. Labovitiadi, Olga Tonnis, Wouter Doro, Francesco Adriaansen, Janik. The sequence listing filed with the application follows.

SEQUENCE LISTING (2 sequences)

SEQ ID NO: 1 - protein, 612 aa, Artificial Sequence
  detoxified exotoxin A of Pseudomonas aeruginosa
AEEAFDLWNECAKACVLDLKDGVRSSRMSVDPAIADTNGQGVLHYSMVLEGGNDALKLAIDNALSITSDGLTIRLEGGVEPNKPVRYSYTRQARGSWSLNWLVPIGHEKPSNIKVFIHELNAGNQLSHMSPIYTIEMGDELLAKLARDATFFVRAHESNEMQPTLAISHAGVSVVMAQAQPRREKRWSEWASGKVLCLLDPLDGVYNYLAQQRCNLDDTWEGKIYRVLAGNPAKHDLDIKPTVISHRLHFPEGGSLAALTAHQACHLPLEAFTRHRQPRGWEQLEQCGYPVQRLVALYLAARLSWNQVDQVIRNALASPGSGGDLGEAIREQPEQARLALTLAAAESERFVRQGTGNDEAGAASADVVSLTCPVAAGECAGPADSGDALLERNYPTGAEFLGDGGDVSFSTRGTQNWTVERLLQAHRQLEERGYVFVGYHGTFLEAAQSIVFGGVRARSQDLDAIWRGFYIAGDPALAYGYAQDQEPDARGRIRNGALLRVYVPRWSLPGFYRTGLTLAAPEAAGEVERLIGHPLPLRLDAITGPEEEGGRVTILGWPLAERTVVIPSAIPTDPRNVGGDLDPSSIPDKEQAISALPDYASQPGKPPREDLK

SEQ ID NO: 2 - protein, 5 aa, Artificial Sequence
  preferred N-linked glycosylation consensus sequence
  MISC_FEATURE (1)..(1): Xaa can be Asp or Glu
  MISC_FEATURE (2)..(2): Xaa can be any amino acid except Pro
  MISC_FEATURE (4)..(4): Xaa can be any amino acid except Pro
  MISC_FEATURE (5)..(5): Xaa can be Ser or Thr
XXNXX